European Patent Specification EP 3 630 968 B1, published May 29, 2024. Title: Tools for Glycan Analysis. Applicant: GENOVIS AB. The sequence listing filed with the application follows.

SEQUENCE LISTING (13 sequences)

SEQ ID NO: 1 - protein, 419 aa, Akkermansia muciniphila
MTWLLCGRGKWNKVKRMMNSVFKCLMSAVCAVALPAFGQEEKTGFPTDRAVTVFSAGEGNPYASIRIPALLSIGKGQLLAFAEGRYKNTDQGENDIIMSVSKNGGKTWSRPRAIAKAHGATFNNPCPVYDAKTRTVTVVFQRYPAGVKERQPNIPDGWDDEKCIRNFMIQSRNGGSSWTKPQEITKTTKRPSGVDIMASGPNAGTQLKSGAHKGRLVIPMNEGPFGKWVISCIYSDDGGKSWKLGQPTANMKGMVNETSIAETDNGGVVMVARHWGAGNCRRIAWSQDGGETWGQVEDAPELFCDSTQNSLMTYSLSDQPAYGGKSRILFSGPSAGRRIKGQVAMSYDNGKTWPVKKLLGEGGFAYSSLAMVEPGIVGVLYEENQEHIKKLKFVPITMEWLTDGEDTGLAPGKKAPVLK

SEQ ID NO: 2 - protein, 381 aa, Akkermansia muciniphila
QEEKTGFPTDRAVTVFSAGEGNPYASIRIPALLSIGKGQLLAFAEGRYKNTDQGENDIIMSVSKNGGKTWSRPRAIAKAHGATFNNPCPVYDAKTRTVTVVFQRYPAGVKERQPNIPDGWDDEKCIRNFMIQSRNGGSSWTKPQEITKTTKRPSGVDIMASGPNAGTQLKSGAHKGRLVIPMNEGPFGKWVISCIYSDDGGKSWKLGQPTANMKGMVNETSIAETDNGGVVMVARHWGAGNCRRIAWSQDGGETWGQVEDAPELFCDSTQNSLMTYSLSDQPAYGGKSRILFSGPSAGRRIKGQVAMSYDNGKTWPVKKLLGEGGFAYSSLAMVEPGIVGVLYEENQEHIKKLKFVPITMEWLTDGEDTGLAPGKKAPVLK

SEQ ID NO: 3 - protein, 393 aa, Artificial Sequence
  sialidase, Am0707 - with additional N terminal methionine and C terminal linker + His6 tag
MQEEKTGFPTDRAVTVFSAGEGNPYASIRIPALLSIGKGQLLAFAEGRYKNTDQGENDIIMSVSKNGGKTWSRPRAIAKAHGATFNNPCPVYDAKTRTVTVVFQRYPAGVKERQPNIPDGWDDEKCIRNFMIQSRNGGSSWTKPQEITKTTKRPSGVDIMASGPNAGTQLKSGAHKGRLVIPMNEGPFGKWVISCIYSDDGGKSWKLGQPTANMKGMVNETSIAETDNGGVVMVARHWGAGNCRRIAWSQDGGETWGQVEDAPELFCDSTQNSLMTYSLSDQPAYGGKSRILFSGPSAGRRIKGQVAMSYDNGKTWPVKKLLGEGGFAYSSLAMVEPGIVGVLYEENQEHIKKLKFVPITMEWLTDGEDTGLAPGKKAPVLKGSGLEHHHHHH

SEQ ID NO: 4 - protein, 595 aa, Akkermansia muciniphila
MKNLLFALLTGSFCCCYAQQKAAPVPEPEVVATPPADAGRGLIRVDSREIRHYSGTRKEPDYLVSRDNGKTWEMKAAPAGYPPNYGGIPKESPAIVRNPLTREFIRVQPIGGFVFLSRGGLDGKWLAVTNDGKLEEDWKDPEKRKNLKKLGGIMRTPVFVNKGRRVIVPFHNMGGGTKFHISDDGGLTWHVSRNGVTSPRHEARPPHQGVRWFNNAVEATVLEMKDGTLWALARTSQDQAWQAFSKDYGETWSKPEPSRFFGTLTMNTLGRLDDGTIVSLWTNTMALPENATAGNGTWEDVFTNRDSHHIAMSGDEGKTWYGFREIILDEHRNHPGYATLDGPEDRGKHQSEMVQLDKNRILISLGQHKNHRRLVIVDRRWVGAKTRATQTGKDLDSQWTIHTYIPQKKGHCSYNRKPSAELVQDPSGGTKKVLQIKRLDDPELVNEKSNVDYRNGGATWNFPNGTTGLVKFRFRVVDGEQADDSGLQVSLTDRLFNACDSTTKDYALFTFPIRLKPAPHLLLGMKKVPFTPGAWHEISLLWQGGQAVVSLDGKKAGTLKMANKSPNGASYIHFISTGSQPDAGILLDTVNARVK

SEQ ID NO: 5 - protein, 577 aa, Akkermansia muciniphila
QQKAAPVPEPEVVATPPADAGRGLIRVDSREIRHYSGTRKEPDYLVSRDNGKTWEMKAAPAGYPPNYGGIPKESPAIVRNPLTREFIRVQPIGGFVFLSRGGLDGKWLAVTNDGKLEEDWKDPEKRKNLKKLGGIMRTPVFVNKGRRVIVPFHNMGGGTKFHISDDGGLTWHVSRNGVTSPRHEARPPHQGVRWFNNAVEATVLEMKDGTLWALARTSQDQAWQAFSKDYGETWSKPEPSRFFGTLTMNTLGRLDDGTIVSLWTNTMALPENATAGNGTWEDVFTNRDSHHIAMSGDEGKTWYGFREIILDEHRNHPGYATLDGPEDRGKHQSEMVQLDKNRILISLGQHKNHRRLVIVDRRWVGAKTRATQTGKDLDSQWTIHTYIPQKKGHCSYNRKPSAELVQDPSGGTKKVLQIKRLDDPELVNEKSNVDYRNGGATWNFPNGTTGLVKFRFRVVDGEQADDSGLQVSLTDRLFNACDSTTKDYALFTFPIRLKPAPHLLLGMKKVPFTPGAWHEISLLWQGGQAVVSLDGKKAGTLKMANKSPNGASYIHFISTGSQPDAGILLDTVNARVK

SEQ ID NO: 6 - protein, 589 aa, Artificial Sequence
  sialidase, Am1757 - with additional N terminal methionine and C terminal linker + His6 tag
MQQKAAPVPEPEVVATPPADAGRGLIRVDSREIRHYSGTRKEPDYLVSRDNGKTWEMKAAPAGYPPNYGGIPKESPAIVRNPLTREFIRVQPIGGFVFLSRGGLDGKWLAVTNDGKLEEDWKDPEKRKNLKKLGGIMRTPVFVNKGRRVIVPFHNMGGGTKFHISDDGGLTWHVSRNGVTSPRHEARPPHQGVRWFNNAVEATVLEMKDGTLWALARTSQDQAWQAFSKDYGETWSKPEPSRFFGTLTMNTLGRLDDGTIVSLWTNTMALPENATAGNGTWEDVFTNRDSHHIAMSGDEGKTWYGFREIILDEHRNHPGYATLDGPEDRGKHQSEMVQLDKNRILISLGQHKNHRRLVIVDRRWVGAKTRATQTGKDLDSQWTIHTYIPQKKGHCSYNRKPSAELVQDPSGGTKKVLQIKRLDDPELVNEKSNVDYRNGGATWNFPNGTTGLVKFRFRVVDGEQADDSGLQVSLTDRLFNACDSTTKDYALFTFPIRLKPAPHLLLGMKKVPFTPGAWHEISLLWQGGQAVVSLDGKKAGTLKMANKSPNGASYIHFISTGSQPDAGILLDTVNARVKGSGLEHHHHHH

SEQ ID NO: 7 - protein, 2122 aa, Streptococcus oralis
MDKRFFEKRCKFSIRKFTLGVASVMIGATFFAASPVLADQARVGSTDNLPSELADLDKKASDEGHDFDKEAAAQNPGSAETTEGPQTEEELLAQEKEKSEKPSNLPKELEDKLEKAEDNGREVDKDQLAQDTGKLVPEDVAKTTNGELNYGATVKIKTPSGEGSGIVVAKDLVLTVSHNFIKDSQEGNIRKVVDNDQGDGDIYSISYPGLPDVKFSKKDIIHWDREGYLKGFKNDLALVRLRTVLENTPVEVTKKPVVKKIGDKLHVFGYPEGKLNPIVNTTVDFAEPYGEGVQGIGYQGGKPGASGGGIFDTEGKLVGVHQNGVVGKRSGGILFSPAQLKWIQDHMQGISSVKPADLEEKEKPAEEKPKEDKPAAAKPETPKAVTPEWQTVANKEQQGTVTIREEKGVRYNQLSSTAQNDNDGKPALFEKQGLTVDANGNATVDLTFKDDSEKGKSRFGVFLKFKDTKNNVFVGYDQGGWFWEYKTPGNSTWYKGNRVAAPEPGSVNRLSITLKSDGQLNASNNDVNLFDTVTLPGAVNENLKNEKKILLKAGTYSNDRTVVSVKTDNQEGVKADDTPAQKETGPAVDDSKVTYDTIQSKVLKAVIDQAFPRVKEYTLNGHTLPGQVQQFNQVFINNHRITPEVTYKKINETTAEYLMKLRDDAHLINAEMTVRLQVVDNQLHFDVTKIVNHNQVTPGQKIDDERKLLSTISFLGNALVSVSSDQAGAKFDGATMSNNTHVSGDDHIDVTNPMKDLAKGYMYGFVSTDKLAAGVWSNSQNSYGGGSNDWTRLTAYKETVGNANYVGIHSSEWQWEKAYKGIVFPEYTKELPSAKVVITEDANADNKVDWQDGAIAYRSIMNNPQGWEKVKDITAYRIAMNFGSQAQNPFLMTLDGIKKINLHTDGLGQGVLLKGYGSEGHDSGHLNYADIGKRIGGVEDFKTLIEKAKKYGAHLGIHVNASETYPESKYFNENILRKNPDGSYSYGWNWLDQGINIDAAYDLAHGRLARWEDLKKKLGEGLDFIYVDVWGNGQSGDNGAWATHVLAKEINKQGWRFAIEWGHGGEYDSTFQHWAADLTYGGYTNKGINSAITRFIRNHQKDSWVGDYRSYGGAANYPLLGGYSMKDFEGWQGRSDYNGYVTNLFAHDVMTKYFQHFTVSKWENGTPVTMTDNGSTYKWTPEMKVELVDAAGNKVVVTRKSNDVNSPQYRERTVTLNGRVIQDGSAYLTPWNWDANGKKLPTEKEKMYYFNTQAGATTWTLPSDWANSKVYLYKLTDQGKTEEQELTVTDGKITLDLLANQPYVLYRSKQTNPEMSWSEGMHIYDQGFNSGTLKHWTISGDASKAEIVKSQGANEMLRIQGNKSKVSLTQKLTGLKPNTKYAVYVGVDNRSNAKASITVNTGEKEVTTYTNKSLALNYIKAYAHNNRRENATVDDTSYFQNMYAFFTTGSDVSNVTLTLSREAGDEATYFDEIRTFENNSSMYGDKHDTGQGTFKQDFENVAQGIFPFVVGGVEGVEDNRTHLSEKHDPYTQRGWNGKKVDDVIEGNWSLKTNGLVSRRNLVYQTIPQNFRFEAGKTYRVTFEYEAGSDNTYAFVVGKGEFQSGRRGTQASNLEMHELPNTWTDSKKAKKVTFLVTGAETGDTWVGIYSTGNASNTRGDAGGNANFRGYNDFMMDNLQIEEITLTGKMLTENALKNYLPTVAMTNYTKESMDALKEAVFNLSQADDDISVEEARAEIAKIEALKNALVQKKTALVAEDFESLDAPAQPGEGLENAFDGNVSSLWHTSWNGGDVGKPATMVLKEPTEITGLRYVPRASDSNGNLRDVKLVVTDESGKEHTFNVTDWPNNNKPKDIDFGKTIKAKKIVLTGTKTYGDGGDKYQSAAELIFTRPQVAETPLDLSGYEAALAKAQKLTDKDNQEEVASVQASMKYATDNHLLTERMVAYFADYLNQLKDSATKPDAPTSSKGEEQPPVLDVPEFKGGVNATEAAVHEVPEFKGGVNAVQALVHELPEYKGGANAVLAAANEVPEYKGGANAVEALVNEKPAYTGVLATAGDQAAPTVEKPEYPLTPSPVADTKTPGAKDEEKLPATGEHSSEVALFLASVSIALSAAVLATKRKEE

SEQ ID NO: 8 - protein, 2084 aa, Streptococcus oralis
DQARVGSTDNLPSELADLDKKASDEGHDFDKEAAAQNPGSAETTEGPQTEEELLAQEKEKSEKPSNLPKELEDKLEKAEDNGREVDKDQLAQDTGKLVPEDVAKTTNGELNYGATVKIKTPSGEGSGIVVAKDLVLTVSHNFIKDSQEGNIRKVVDNDQGDGDIYSISYPGLPDVKFSKKDIIHWDREGYLKGFKNDLALVRLRTVLENTPVEVTKKPVVKKIGDKLHVFGYPEGKLNPIVNTTVDFAEPYGEGVQGIGYQGGKPGASGGGIFDTEGKLVGVHQNGVVGKRSGGILFSPAQLKWIQDHMQGISSVKPADLEEKEKPAEEKPKEDKPAAAKPETPKAVTPEWQTVANKEQQGTVTIREEKGVRYNQLSSTAQNDNDGKPALFEKQGLTVDANGNATVDLTFKDDSEKGKSRFGVFLKFKDTKNNVFVGYDQGGWFWEYKTPGNSTWYKGNRVAAPEPGSVNRLSITLKSDGQLNASNNDVNLFDTVTLPGAVNENLKNEKKILLKAGTYSNDRTVVSVKTDNQEGVKADDTPAQKETGPAVDDSKVTYDTIQSKVLKAVIDQAFPRVKEYTLNGHTLPGQVQQFNQVFINNHRITPEVTYKKINETTAEYLMKLRDDAHLINAEMTVRLQVVDNQLHFDVTKIVNHNQVTPGQKIDDERKLLSTISFLGNALVSVSSDQAGAKFDGATMSNNTHVSGDDHIDVTNPMKDLAKGYMYGFVSTDKLAAGVWSNSQNSYGGGSNDWTRLTAYKETVGNANYVGIHSSEWQWEKAYKGIVFPEYTKELPSAKVVITEDANADNKVDWQDGAIAYRSIMNNPQGWEKVKDITAYRIAMNFGSQAQNPFLMTLDGIKKINLHTDGLGQGVLLKGYGSEGHDSGHLNYADIGKRIGGVEDFKTLIEKAKKYGAHLGIHVNASETYPESKYFNENILRKNPDGSYSYGWNWLDQGINIDAAYDLAHGRLARWEDLKKKLGEGLDFIYVDVWGNGQSGDNGAWATHVLAKEINKQGWRFAIEWGHGGEYDSTFQHWAADLTYGGYTNKGINSAITRFIRNHQKDSWVGDYRSYGGAANYPLLGGYSMKDFEGWQGRSDYNGYVTNLFAHDVMTKYFQHFTVSKWENGTPVTMTDNGSTYKWTPEMKVELVDAAGNKVVVTRKSNDVNSPQYRERTVTLNGRVIQDGSAYLTPWNWDANGKKLPTEKEKMYYFNTQAGATTWTLPSDWANSKVYLYKLTDQGKTEEQELTVTDGKITLDLLANQPYVLYRSKQTNPEMSWSEGMHIYDQGFNSGTLKHWTISGDASKAEIVKSQGANEMLRIQGNKSKVSLTQKLTGLKPNTKYAVYVGVDNRSNAKASITVNTGEKEVTTYTNKSLALNYIKAYAHNNRRENATVDDTSYFQNMYAFFTTGSDVSNVTLTLSREAGDEATYFDEIRTFENNSSMYGDKHDTGQGTFKQDFENVAQGIFPFVVGGVEGVEDNRTHLSEKHDPYTQRGWNGKKVDDVIEGNWSLKTNGLVSRRNLVYQTIPQNFRFEAGKTYRVTFEYEAGSDNTYAFVVGKGEFQSGRRGTQASNLEMHELPNTWTDSKKAKKVTFLVTGAETGDTWVGIYSTGNASNTRGDAGGNANFRGYNDFMMDNLQIEEITLTGKMLTENALKNYLPTVAMTNYTKESMDALKEAVFNLSQADDDISVEEARAEIAKIEALKNALVQKKTALVAEDFESLDAPAQPGEGLENAFDGNVSSLWHTSWNGGDVGKPATMVLKEPTEITGLRYVPRASDSNGNLRDVKLVVTDESGKEHTFNVTDWPNNNKPKDIDFGKTIKAKKIVLTGTKTYGDGGDKYQSAAELIFTRPQVAETPLDLSGYEAALAKAQKLTDKDNQEEVASVQASMKYATDNHLLTERMVAYFADYLNQLKDSATKPDAPTSSKGEEQPPVLDVPEFKGGVNATEAAVHEVPEFKGGVNAVQALVHELPEYKGGANAVLAAANEVPEYKGGANAVEALVNEKPAYTGVLATAGDQAAPTVEKPEYPLTPSPVADTKTPGAKDEEKLPATGEHSSEVALFLASVSIALSAAVLATKRKEE

SEQ ID NO: 9 - protein, 2053 aa, Streptococcus oralis
DQARVGSTDNLPSELADLDKKASDEGHDFDKEAAAQNPGSAETTEGPQTEEELLAQEKEKSEKPSNLPKELEDKLEKAEDNGREVDKDQLAQDTGKLVPEDVAKTTNGELNYGATVKIKTPSGEGSGIVVAKDLVLTVSHNFIKDSQEGNIRKVVDNDQGDGDIYSISYPGLPDVKFSKKDIIHWDREGYLKGFKNDLALVRLRTVLENTPVEVTKKPVVKKIGDKLHVFGYPEGKLNPIVNTTVDFAEPYGEGVQGIGYQGGKPGASGGGIFDTEGKLVGVHQNGVVGKRSGGILFSPAQLKWIQDHMQGISSVKPADLEEKEKPAEEKPKEDKPAAAKPETPKAVTPEWQTVANKEQQGTVTIREEKGVRYNQLSSTAQNDNDGKPALFEKQGLTVDANGNATVDLTFKDDSEKGKSRFGVFLKFKDTKNNVFVGYDQGGWFWEYKTPGNSTWYKGNRVAAPEPGSVNRLSITLKSDGQLNASNNDVNLFDTVTLPGAVNENLKNEKKILLKAGTYSNDRTVVSVKTDNQEGVKADDTPAQKETGPAVDDSKVTYDTIQSKVLKAVIDQAFPRVKEYTLNGHTLPGQVQQFNQVFINNHRITPEVTYKKINETTAEYLMKLRDDAHLINAEMTVRLQVVDNQLHFDVTKIVNHNQVTPGQKIDDERKLLSTISFLGNALVSVSSDQAGAKFDGATMSNNTHVSGDDHIDVTNPMKDLAKGYMYGFVSTDKLAAGVWSNSQNSYGGGSNDWTRLTAYKETVGNANYVGIHSSEWQWEKAYKGIVFPEYTKELPSAKVVITEDANADNKVDWQDGAIAYRSIMNNPQGWEKVKDITAYRIAMNFGSQAQNPFLMTLDGIKKINLHTDGLGQGVLLKGYGSEGHDSGHLNYADIGKRIGGVEDFKTLIEKAKKYGAHLGIHVNASETYPESKYFNENILRKNPDGSYSYGWNWLDQGINIDAAYDLAHGRLARWEDLKKKLGEGLDFIYVDVWGNGQSGDNGAWATHVLAKEINKQGWRFAIEWGHGGEYDSTFQHWAADLTYGGYTNKGINSAITRFIRNHQKDSWVGDYRSYGGAANYPLLGGYSMKDFEGWQGRSDYNGYVTNLFAHDVMTKYFQHFTVSKWENGTPVTMTDNGSTYKWTPEMKVELVDAAGNKVVVTRKSNDVNSPQYRERTVTLNGRVIQDGSAYLTPWNWDANGKKLPTEKEKMYYFNTQAGATTWTLPSDWANSKVYLYKLTDQGKTEEQELTVTDGKITLDLLANQPYVLYRSKQTNPEMSWSEGMHIYDQGFNSGTLKHWTISGDASKAEIVKSQGANEMLRIQGNKSKVSLTQKLTGLKPNTKYAVYVGVDNRSNAKASITVNTGEKEVTTYTNKSLALNYIKAYAHNNRRENATVDDTSYFQNMYAFFTTGSDVSNVTLTLSREAGDEATYFDEIRTFENNSSMYGDKHDTGQGTFKQDFENVAQGIFPFVVGGVEGVEDNRTHLSEKHDPYTQRGWNGKKVDDVIEGNWSLKTNGLVSRRNLVYQTIPQNFRFEAGKTYRVTFEYEAGSDNTYAFVVGKGEFQSGRRGTQASNLEMHELPNTWTDSKKAKKVTFLVTGAETGDTWVGIYSTGNASNTRGDAGGNANFRGYNDFMMDNLQIEEITLTGKMLTENALKNYLPTVAMTNYTKESMDALKEAVFNLSQADDDISVEEARAEIAKIEALKNALVQKKTALVAEDFESLDAPAQPGEGLENAFDGNVSSLWHTSWNGGDVGKPATMVLKEPTEITGLRYVPRASDSNGNLRDVKLVVTDESGKEHTFNVTDWPNNNKPKDIDFGKTIKAKKIVLTGTKTYGDGGDKYQSAAELIFTRPQVAETPLDLSGYEAALAKAQKLTDKDNQEEVASVQASMKYATDNHLLTERMVAYFADYLNQLKDSATKPDAPTSSKGEEQPPVLDVPEFKGGVNATEAAVHEVPEFKGGVNAVQALVHELPEYKGGANAVLAAANEVPEYKGGANAVEALVNEKPAYTGVLATAGDQAAPTVEKPEYPLTPSPVADTKTPGAKDEEKLPA

SEQ ID NO: 10 - protein, 2065 aa, Artificial Sequence
  O-glycosidase from S. oralis with additional N terminal Met, C terminal GSGLE-His6tag, and signal sequence and C terminal element of LPXTG cell wall anchor motif removed
MDQARVGSTDNLPSELADLDKKASDEGHDFDKEAAAQNPGSAETTEGPQTEEELLAQEKEKSEKPSNLPKELEDKLEKAEDNGREVDKDQLAQDTGKLVPEDVAKTTNGELNYGATVKIKTPSGEGSGIVVAKDLVLTVSHNFIKDSQEGNIRKVVDNDQGDGDIYSISYPGLPDVKFSKKDIIHWDREGYLKGFKNDLALVRLRTVLENTPVEVTKKPVVKKIGDKLHVFGYPEGKLNPIVNTTVDFAEPYGEGVQGIGYQGGKPGASGGGIFDTEGKLVGVHQNGVVGKRSGGILFSPAQLKWIQDHMQGISSVKPADLEEKEKPAEEKPKEDKPAAAKPETPKAVTPEWQTVANKEQQGTVTIREEKGVRYNQLSSTAQNDNDGKPALFEKQGLTVDANGNATVDLTFKDDSEKGKSRFGVFLKFKDTKNNVFVGYDQGGWFWEYKTPGNSTWYKGNRVAAPEPGSVNRLSITLKSDGQLNASNNDVNLFDTVTLPGAVNENLKNEKKILLKAGTYSNDRTVVSVKTDNQEGVKADDTPAQKETGPAVDDSKVTYDTIQSKVLKAVIDQAFPRVKEYTLNGHTLPGQVQQFNQVFINNHRITPEVTYKKINETTAEYLMKLRDDAHLINAEMTVRLQVVDNQLHFDVTKIVNHNQVTPGQKIDDERKLLSTISFLGNALVSVSSDQAGAKFDGATMSNNTHVSGDDHIDVTNPMKDLAKGYMYGFVSTDKLAAGVWSNSQNSYGGGSNDWTRLTAYKETVGNANYVGIHSSEWQWEKAYKGIVFPEYTKELPSAKVVITEDANADNKVDWQDGAIAYRSIMNNPQGWEKVKDITAYRIAMNFGSQAQNPFLMTLDGIKKINLHTDGLGQGVLLKGYGSEGHDSGHLNYADIGKRIGGVEDFKTLIEKAKKYGAHLGIHVNASETYPESKYFNENILRKNPDGSYSYGWNWLDQGINIDAAYDLAHGRLARWEDLKKKLGEGLDFIYVDVWGNGQSGDNGAWATHVLAKEINKQGWRFAIEWGHGGEYDSTFQHWAADLTYGGYTNKGINSAITRFIRNHQKDSWVGDYRSYGGAANYPLLGGYSMKDFEGWQGRSDYNGYVTNLFAHDVMTKYFQHFTVSKWENGTPVTMTDNGSTYKWTPEMKVELVDAAGNKVVVTRKSNDVNSPQYRERTVTLNGRVIQDGSAYLTPWNWDANGKKLPTEKEKMYYFNTQAGATTWTLPSDWANSKVYLYKLTDQGKTEEQELTVTDGKITLDLLANQPYVLYRSKQTNPEMSWSEGMHIYDQGFNSGTLKHWTISGDASKAEIVKSQGANEMLRIQGNKSKVSLTQKLTGLKPNTKYAVYVGVDNRSNAKASITVNTGEKEVTTYTNKSLALNYIKAYAHNNRRENATVDDTSYFQNMYAFFTTGSDVSNVTLTLSREAGDEATYFDEIRTFENNSSMYGDKHDTGQGTFKQDFENVAQGIFPFVVGGVEGVEDNRTHLSEKHDPYTQRGWNGKKVDDVIEGNWSLKTNGLVSRRNLVYQTIPQNFRFEAGKTYRVTFEYEAGSDNTYAFVVGKGEFQSGRRGTQASNLEMHELPNTWTDSKKAKKVTFLVTGAETGDTWVGIYSTGNASNTRGDAGGNANFRGYNDFMMDNLQIEEITLTGKMLTENALKNYLPTVAMTNYTKESMDALKEAVFNLSQADDDISVEEARAEIAKIEALKNALVQKKTALVAEDFESLDAPAQPGEGLENAFDGNVSSLWHTSWNGGDVGKPATMVLKEPTEITGLRYVPRASDSNGNLRDVKLVVTDESGKEHTFNVTDWPNNNKPKDIDFGKTIKAKKIVLTGTKTYGDGGDKYQSAAELIFTRPQVAETPLDLSGYEAALAKAQKLTDKDNQEEVASVQASMKYATDNHLLTERMVAYFADYLNQLKDSATKPDAPTSSKGEEQPPVLDVPEFKGGVNATEAAVHEVPEFKGGVNAVQALVHELPEYKGGANAVLAAANEVPEYKGGANAVEALVNEKPAYTGVLATAGDQAAPTVEKPEYPLTPSPVADTKTPGAKDEEKLPAGSGLEHHHHHH

SEQ ID NO: 11 - protein, 361 aa, Akkermansia muciniphila
EVTVPDALKDRIALKKTARQLNIVYFLGSDTEPVPDYERRLSELLLYLQQFYGKEMQRHGYGARSFGLDIKSPGRVNIIEYKAKNPAAHYPYENGGGWKAAQELDEFFKAHPDRKKSQHTLIIMPTWNDEKNGPDNPGGVPFYGMGRNCFALDYPAFDIKHLGQKTREGRLLTKWYGGMAHELGHGLNLPHNHQTASDGKKYGTALMGSGNYTFGTSPTFLTPASCALLDACEVFSVTPSQQFYEGKPEVEVGDVAISFKGDQILVSGNYKSPQTVKALNVYIQDPPYAVNQDYDAVSFSRRLGKKSGKFSMKIDKKELEGLNNNEFRISLMFILANGLHMQKHFTFHWDALQDYRDGSKS

SEQ ID NO: 12 - protein, 371 aa, Artificial Sequence
  O-glycoprotein-specific endoprotease (LS)
MEVTVPDALKDRIALKKTARQLNIVYFLGSDTEPVPDYERRLSELLLYLQQFYGKEMQRHGYGARSFGLDIKSPGRVNIIEYKAKNPAAHYPYENGGGWKAAQELDEFFKAHPDRKKSQHTLIIMPTWNDEKNGPDNPGGVPFYGMGRNCFALDYPAFDIKHLGQKTREGRLLTKWYGGMAHELGHGLNLPHNHQTASDGKKYGTALMGSGNYTFGTSPTFLTPASCALLDACEVFSVTPSQQFYEGKPEVEVGDVAISFKGDQILVSGNYKSPQTVKALNVYIQDPPYAVNQDYDAVSFSRRLGKKSGKFSMKIDKKELEGLNNNEFRISLMFILANGLHMQKHFTFHWDALQDYRDGSKSGSGHHHHHH

SEQ ID NO: 13 - DNA, 6198 bp, Artificial Sequence
  Nucleotide encoding O-glycosidase from S. oralis (additional N terminal Met, C terminal GSGLE-His6tag, and signal sequence and C terminal element of LPXTG cell wall anchor motif removed)
atggaccaagcgcgtgtgggtagcaccgataacctgccgagcgagctggcggatctggacaagaaagcgagcgacgaaggccacgattttgacaaagaggcggcggcgcagaacccgggtagcgcggaaaccaccgaaggtccgcagaccgaggaagagctgctggcgcaagaaaaagagaagagcgagaagccgagcaacctgccgaaagaactggaggataaactggaaaaggcggaggacaacggtcgtgaagtggataaagaccagctggcgcaagacaccggcaagctggtgccggaggatgttgcgaaaaccaccaacggtgaactgaactacggcgcgaccgttaaaattaagaccccgagcggcgagggtagcggtattgtggttgcgaaggacctggtgctgaccgttagccacaacttcattaaggatagccaggaaggtaatatccgtaaagtggttgataacgaccaaggcgatggtgacatctacagcattagctatccgggcctgccggacgttaagttcagcaagaaagatatcatccactgggaccgtgagggttacctgaaaggcttcaagaacgatctggcgctggtgcgtctgcgtaccgttctggaaaacaccccggttgaggtgaccaagaaaccggtggttaagaaaattggtgacaagctgcacgtgtttggttatccggagggcaaactgaacccgatcgtgaacaccaccgttgatttcgcggaaccgtacggcgagggtgttcagggcattggttatcaaggtggcaaaccgggcgcgagcggtggcggtatctttgacaccgaaggcaagctggttggcgtgcaccagaacggtgtggttggcaaacgtagcggcggtattctgttcagcccggcgcaactgaagtggattcaggaccacatgcaaggtatcagcagcgtgaaaccggcggatctggaagagaaagagaagccggcggaagagaaaccgaaggaagacaagccggcggcggcgaagccggaaaccccgaaagcggttaccccggagtggcaaaccgtggcgaacaaggaacagcaaggtaccgttaccatccgtgaagagaaaggcgtgcgttacaaccagctgagcagcaccgcgcaaaacgataacgacggcaagccggcgctgtttgagaaacagggtctgaccgttgacgcgaacggcaacgcgaccgtggatctgaccttcaaggacgatagcgaaaaaggcaagagccgtttcggcgtttttctgaaattcaaggacaccaaaaacaacgtttttgtgggttacgatcaaggcggttggttctgggagtataagaccccgggtaacagcacctggtacaagggtaaccgtgtggcggcgccggaaccgggtagcgtgaaccgtctgagcattaccctgaaaagcgacggccagctgaacgcgagcaacaacgatgtgaacctgttcgacaccgttaccctgccgggtgcggtgaacgaaaacctgaagaacgagaagaaaatcctgctgaaagcgggcacctacagcaacgaccgtaccgtggttagcgttaagaccgataaccaggaaggtgtgaaagcggacgataccccggcgcaaaaggaaaccggtccggcggtggacgatagcaaggttacctacgacaccattcagagcaaagtgctgaaggcggttatcgatcaagcgtttccgcgtgtgaaagagtataccctgaacggtcacaccctgccgggtcaggttcagcaatttaaccaagtgttcattaacaaccaccgtatcaccccggaagtgacctataagaaaattaacgaaaccaccgcggagtacctgatgaagctgcgtgacgatgcgcacctgatcaacgcggaaatgaccgtgcgtctgcaggtggttgataaccaactgcacttcgacgtgaccaaaattgttaaccacaaccaggttaccccgggtcaaaagattgacgatgagcgtaaactgctgagcaccatcagctttctgggcaacgcgctggttagcgtgagcagcgatcaagcgggtgcgaagtttgatggtgcgaccatgagcaacaacacccacgttagcggtgacgatcacatcgatgtgaccaacccgatgaaagacctggcgaagggttacatgtatggctttgttagcaccgacaagctggcggcgggtgtgtggagcaacagccaaaacagctacggcggtggcagcaacgattggacccgtctgaccgcgtataaagaaaccgttggtaacgcgaactacgtgggcattcacagcagcgaatggcagtgggagaaagcgtacaagggtatcgtgttcccggaatataccaaggagctgccgagcgcgaaagtggttatcaccgaggatgcgaacgcggacaacaaagtggattggcaggacggtgcgattgcgtaccgtagcatcatgaacaacccgcaaggctgggaaaaagttaaggacattaccgcgtatcgtatcgcgatgaactttggtagccaggcgcaaaacccgttcctgatgaccctggacggcatcaagaaaattaacctgcacaccgatggcctgggtcagggcgttctgctgaagggttatggtagcgagggtcatgacagcggtcacctgaactacgcggatatcggtaaacgtattggtggcgtggaagactttaagaccctgattgagaaagcgaagaaatacggtgcgcacctgggcatccacgttaacgcgagcgaaacctacccggagagcaagtatttcaacgaaaacattctgcgtaaaaacccggacggtagctacagctatggctggaactggctggatcagggtatcaacattgatgcggcgtacgacctggcgcatggccgtctggcgcgttgggaggacctgaagaaaaagctgggtgaaggcctggattttatctatgttgacgtgtggggtaacggtcagagcggtgataacggtgcgtgggcgacccatgtgctggcgaaagagattaacaagcaaggttggcgttttgcgatcgaatggggccacggtggcgagtacgacagcaccttccagcactgggcggcggatctgacctacggtggctataccaacaagggtatcaacagcgcgattacccgtttcatccgtaaccaccagaaagatagctgggttggcgactaccgtagctatggtggcgcggcgaactacccgctgctgggtggctatagcatgaaggactttgagggttggcaaggccgtagcgattacaacggttatgttaccaacctgttcgcgcacgacgtgatgaccaagtactttcagcacttcaccgttagcaaatgggaaaacggtaccccggtgaccatgaccgataacggcagcacctataagtggaccccggaaatgaaagtggagctggttgacgcggcgggtaacaaggtggttgtgacccgtaaaagcaacgatgtgaacagcccgcagtaccgtgagcgtaccgttaccctgaacggtcgtgtgatccaagacggcagcgcgtatctgaccccgtggaactgggatgcgaacggtaaaaagctgccgaccgaaaaagagaagatgtactattttaacacccaagcgggtgcgaccacctggaccctgccgagcgactgggcgaacagcaaggtttacctgtataaactgaccgatcagggcaagaccgaggagcaagaactgaccgtgaccgatggcaaaattaccctggacctgctggcgaaccagccgtacgttctgtatcgtagcaagcaaaccaacccggaaatgagctggagcgagggtatgcacatctacgaccaaggtttcaacagcggcaccctgaaacactggaccattagcggcgatgcgagcaaggcggagatcgtgaaaagccagggtgcgaacgaaatgctgcgtatccaaggcaacaaaagcaaggttagcctgacccagaagctgaccggtctgaaaccgaacaccaagtacgcggtttatgtgggcgttgacaaccgtagcaacgcgaaagcgagcattaccgttaacaccggtgaaaaagaggtgaccacctacaccaacaagagcctggcgctgaactacatcaaagcgtatgcgcacaacaaccgtcgtgagaacgcgaccgtggacgataccagctacttccagaacatgtatgcgttctttaccaccggtagcgacgtgagcaacgttaccctgaccctgagccgtgaagcgggcgatgaggcgacctattttgacgaaattcgtaccttcgagaacaacagcagcatgtacggtgataagcacgacaccggtcagggcacctttaaacaagatttcgaaaacgttgcgcaaggtatcttcccgtttgttgtgggtggcgtggaaggcgttgaggacaaccgtacccacctgagcgagaagcacgatccgtacacccagcgtggttggaacggcaaaaaggtggacgatgttattgagggtaactggagcctgaaaaccaacggcctggttagccgtcgtaacctggtgtaccagaccatcccgcaaaacttccgttttgaggcgggcaagacctaccgtgtgacctttgaatatgaggcgggcagcgacaacacctatgcgtttgttgtgggtaaaggcgaattccagagcggtcgtcgtggcacccaagcgagcaacctggaaatgcacgagctgccgaacacctggaccgatagcaaaaaggcgaaaaaggtgaccttcctggttaccggtgcggaaaccggtgacacctgggtgggtatctacagcaccggcaacgcgagcaacacccgtggtgatgcgggtggcaacgcgaactttcgtggctataacgatttcatgatggacaacctgcaaatcgaagagattaccctgaccggcaagatgctgaccgaaaacgcgctgaaaaactatctgccgaccgttgcgatgaccaactacaccaaggaaagcatggacgcgctgaaagaggcggttttcaacctgagccaggcggacgatgacatcagcgtggaagaggcgcgtgcggaaatcgcgaagattgaggcgctgaaaaacgcgctggttcagaaaaagaccgcgctggttgcggaagattttgagagcctggatgcgccggcgcaaccgggtgaaggcctggagaacgcgttcgacggtaacgttagcagcctgtggcacaccagctggaacggtggcgatgttggcaagccggcgaccatggtgctgaaagaaccgaccgagatcaccggtctgcgttatgtgccgcgtgcgagcgatagcaacggcaacctgcgtgacgttaagctggttgtgaccgatgaaagcggtaaagagcacacctttaacgtgaccgactggccgaacaacaacaaaccgaaggatattgacttcggcaaaaccattaaggcgaaaaagatcgttctgaccggtaccaagacctacggcgatggtggcgacaaatatcagagcgcggcggagctgatctttacccgtccgcaagtggcggaaaccccgctggatctgagcggttacgaagcggcgctggcgaaagcgcagaagctgaccgataaggacaaccaggaagaggtggcgagcgttcaagcgagcatgaaatatgcgaccgacaaccacctgctgaccgaacgtatggttgcgtacttcgcggattatctgaaccaactgaaggatagcgcgaccaaaccggatgcgccgaccagcagcaagggtgaagaacagccgccggtgctggatgttccggagtttaaaggtggcgtgaacgcgaccgaggcggcggtgcacgaagttccggagttcaagggtggcgtgaacgcggttcaggcgctggttcacgaactgccggagtataaaggtggcgcgaacgcggttctggcggcggcgaacgaagtgccggagtacaagggtggcgcgaacgcggtggaagcgctggttaacgagaaaccggcgtataccggtgttctggcgaccgcgggcgaccaggcggcgccgaccgtggaaaaaccggagtacccgctgaccccgagcccggttgcggacaccaaaaccccgggtgcgaaagatgaagagaagctgccggcgggtagcggcctcgagcaccaccaccaccaccactga